European Patent Application EP 4 717 715 A1, published April 1, 2026. Title: 一种腺相关病毒衣壳蛋白、包含其的腺相关病毒、载体及应用. Applicant: 北京因诺惟康医药科技有限公司. The sequence listing filed with the application follows.

SEQUENCE LISTING (66 sequences)

SEQ ID NO: 1 - protein, 12 aa, synthetic construct
AAARGDLATIAA

SEQ ID NO: 2 - protein, 12 aa, synthetic construct
AAARGDLGRLAA

SEQ ID NO: 3 - protein, 12 aa, synthetic construct
AAARGDLQNIAA

SEQ ID NO: 4 - protein, 12 aa, synthetic construct
AAARGDLQNLAA

SEQ ID NO: 5 - protein, 12 aa, synthetic construct
AAARGDLAAIAA

SEQ ID NO: 6 - protein, 12 aa, synthetic construct
AAARGDLATLAA

SEQ ID NO: 7 - protein, 12 aa, synthetic construct
AAARGDLATPAA

SEQ ID NO: 8 - protein, 12 aa, synthetic construct
AAARGDLGRPAA

SEQ ID NO: 9 - protein, 12 aa, synthetic construct
AAARGDLGTLAA

SEQ ID NO: 10 - protein, 12 aa, synthetic construct
AAARGDLARIAA

SEQ ID NO: 11 - protein, 12 aa, synthetic construct
AAARGSLQNIAA

SEQ ID NO: 12 - protein, 12 aa, synthetic construct
AAARGSLQNLAA

SEQ ID NO: 13 - protein, 9 aa, synthetic construct
AAARGSLAA

SEQ ID NO: 14 - protein, 12 aa, synthetic construct
AAAGNGRAHAAA

SEQ ID NO: 15 - protein, 747 aa, synthetic construct
MAADGYLPDWLEDTLSEGIRQWWKLKPGPPPPKPAERHKDDSRGLVLPGYKYLGPFNGLDKGEPVNEADAAALEHDKAYDRQLDSGDNPYLKYNHADAEFQERLKEDTSFGGNLGRAVFQAKKRVLEPLGLVEEPVKTAPGKKRPVEHSPVEPDSSSGTGKAGQQPARKRLNFGQTGDADSVPDPQPLGQPPAAPSGLGTNTMATGSGAPMADNNEGADGVGNSSGNWHCDSTWMGDRVITTSTRTWALPTYNNHLYKQISSQSGASNDNHYFGYSTPWGYFDFNRFHCHFSPRDWQRLINNNWGFRPKRLNFKLFNIQVKEVTQNDGTTTIANNLTSTVQVFTDSEYQLPYVLGSAHQGCLPPFPADVFMVPQYGYLTLNNGSQAVGRSSFYCLEYFPSQMLRTGNNFTFSYTFEDVPFHSSYAHSQSLDRLMNPLIDQYLYYLSRTNTPSGTTTQSRLQFSQAGASDIRDQSRNWLPGPCYRQQRVSKTSADNNNSEYSWTGATKYHLNGRDSLVNPGPAMASHKDDEEKFFPQSGVLIFGKQGSEKTNVDIEKVMITDEEEIRTTNPVATEQYGSVSTNLQRGNAAARGDLATIAARQAATADVNTQGVLPGMVWQDRDVYLQGPIWAKIPHTDGHFHPSPLMGGFGLKHPPPQILIKNTPVPANPSTTFSAAKFASFITQYSTGQVSVEIEWELQKENSKRWNPEIQYTSNYNKSVNVDFTVDTNGVYSEPRPIGTRYLTRNL

SEQ ID NO: 16 - protein, 747 aa, synthetic construct
MAADGYLPDWLEDTLSEGIRQWWKLKPGPPPPKPAERHKDDSRGLVLPGYKYLGPFNGLDKGEPVNEADAAALEHDKAYDRQLDSGDNPYLKYNHADAEFQERLKEDTSFGGNLGRAVFQAKKRVLEPLGLVEEPVKTAPGKKRPVEHSPVEPDSSSGTGKAGQQPARKRLNFGQTGDADSVPDPQPLGQPPAAPSGLGTNTMATGSGAPMADNNEGADGVGNSSGNWHCDSTWMGDRVITTSTRTWALPTYNNHLYKQISSQSGASNDNHYFGYSTPWGYFDFNRFHCHFSPRDWQRLINNNWGFRPKRLNFKLFNIQVKEVTQNDGTTTIANNLTSTVQVFTDSEYQLPYVLGSAHQGCLPPFPADVFMVPQYGYLTLNNGSQAVGRSSFYCLEYFPSQMLRTGNNFTFSYTFEDVPFHSSYAHSQSLDRLMNPLIDQYLYYLSRTNTPSGTTTQSRLQFSQAGASDIRDQSRNWLPGPCYRQQRVSKTSADNNNSEYSWTGATKYHLNGRDSLVNPGPAMASHKDDEEKFFPQSGVLIFGKQGSEKTNVDIEKVMITDEEEIRTTNPVATEQYGSVSTNLQRGNAAARGDLGRLAARQAATADVNTQGVLPGMVWQDRDVYLQGPIWAKIPHTDGHFHPSPLMGGFGLKHPPPQILIKNTPVPANPSTTFSAAKFASFITQYSTGQVSVEIEWELQKENSKRWNPEIQYTSNYNKSVNVDFTVDTNGVYSEPRPIGTRYLTRNL

SEQ ID NO: 17 - protein, 747 aa, synthetic construct
MAADGYLPDWLEDTLSEGIRQWWKLKPGPPPPKPAERHKDDSRGLVLPGYKYLGPFNGLDKGEPVNEADAAALEHDKAYDRQLDSGDNPYLKYNHADAEFQERLKEDTSFGGNLGRAVFQAKKRVLEPLGLVEEPVKTAPGKKRPVEHSPVEPDSSSGTGKAGQQPARKRLNFGQTGDADSVPDPQPLGQPPAAPSGLGTNTMATGSGAPMADNNEGADGVGNSSGNWHCDSTWMGDRVITTSTRTWALPTYNNHLYKQISSQSGASNDNHYFGYSTPWGYFDFNRFHCHFSPRDWQRLINNNWGFRPKRLNFKLFNIQVKEVTQNDGTTTIANNLTSTVQVFTDSEYQLPYVLGSAHQGCLPPFPADVFMVPQYGYLTLNNGSQAVGRSSFYCLEYFPSQMLRTGNNFTFSYTFEDVPFHSSYAHSQSLDRLMNPLIDQYLYYLSRTNTPSGTTTQSRLQFSQAGASDIRDQSRNWLPGPCYRQQRVSKTSADNNNSEYSWTGATKYHLNGRDSLVNPGPAMASHKDDEEKFFPQSGVLIFGKQGSEKTNVDIEKVMITDEEEIRTTNPVATEQYGSVSTNLQRGNAAARGDLQNIAARQAATADVNTQGVLPGMVWQDRDVYLQGPIWAKIPHTDGHFHPSPLMGGFGLKHPPPQILIKNTPVPANPSTTFSAAKFASFITQYSTGQVSVEIEWELQKENSKRWNPEIQYTSNYNKSVNVDFTVDTNGVYSEPRPIGTRYLTRNL

SEQ ID NO: 18 - protein, 747 aa, synthetic construct
MAADGYLPDWLEDTLSEGIRQWWKLKPGPPPPKPAERHKDDSRGLVLPGYKYLGPFNGLDKGEPVNEADAAALEHDKAYDRQLDSGDNPYLKYNHADAEFQERLKEDTSFGGNLGRAVFQAKKRVLEPLGLVEEPVKTAPGKKRPVEHSPVEPDSSSGTGKAGQQPARKRLNFGQTGDADSVPDPQPLGQPPAAPSGLGTNTMATGSGAPMADNNEGADGVGNSSGNWHCDSTWMGDRVITTSTRTWALPTYNNHLYKQISSQSGASNDNHYFGYSTPWGYFDFNRFHCHFSPRDWQRLINNNWGFRPKRLNFKLFNIQVKEVTQNDGTTTIANNLTSTVQVFTDSEYQLPYVLGSAHQGCLPPFPADVFMVPQYGYLTLNNGSQAVGRSSFYCLEYFPSQMLRTGNNFTFSYTFEDVPFHSSYAHSQSLDRLMNPLIDQYLYYLSRTNTPSGTTTQSRLQFSQAGASDIRDQSRNWLPGPCYRQQRVSKTSADNNNSEYSWTGATKYHLNGRDSLVNPGPAMASHKDDEEKFFPQSGVLIFGKQGSEKTNVDIEKVMITDEEEIRTTNPVATEQYGSVSTNLQRGNAAARGDLQNLAARQAATADVNTQGVLPGMVWQDRDVYLQGPIWAKIPHTDGHFHPSPLMGGFGLKHPPPQILIKNTPVPANPSTTFSAAKFASFITQYSTGQVSVEIEWELQKENSKRWNPEIQYTSNYNKSVNVDFTVDTNGVYSEPRPIGTRYLTRNL

SEQ ID NO: 19 - protein, 747 aa, synthetic construct
MAADGYLPDWLEDTLSEGIRQWWKLKPGPPPPKPAERHKDDSRGLVLPGYKYLGPFNGLDKGEPVNEADAAALEHDKAYDRQLDSGDNPYLKYNHADAEFQERLKEDTSFGGNLGRAVFQAKKRVLEPLGLVEEPVKTAPGKKRPVEHSPVEPDSSSGTGKAGQQPARKRLNFGQTGDADSVPDPQPLGQPPAAPSGLGTNTMATGSGAPMADNNEGADGVGNSSGNWHCDSTWMGDRVITTSTRTWALPTYNNHLYKQISSQSGASNDNHYFGYSTPWGYFDFNRFHCHFSPRDWQRLINNNWGFRPKRLNFKLFNIQVKEVTQNDGTTTIANNLTSTVQVFTDSEYQLPYVLGSAHQGCLPPFPADVFMVPQYGYLTLNNGSQAVGRSSFYCLEYFPSQMLRTGNNFTFSYTFEDVPFHSSYAHSQSLDRLMNPLIDQYLYYLSRTNTPSGTTTQSRLQFSQAGASDIRDQSRNWLPGPCYRQQRVSKTSADNNNSEYSWTGATKYHLNGRDSLVNPGPAMASHKDDEEKFFPQSGVLIFGKQGSEKTNVDIEKVMITDEEEIRTTNPVATEQYGSVSTNLQRGNAAARGDLAAIAARQAATADVNTQGVLPGMVWQDRDVYLQGPIWAKIPHTDGHFHPSPLMGGFGLKHPPPQILIKNTPVPANPSTTFSAAKFASFITQYSTGQVSVEIEWELQKENSKRWNPEIQYTSNYNKSVNVDFTVDTNGVYSEPRPIGTRYLTRNL

SEQ ID NO: 20 - protein, 747 aa, synthetic construct
MAADGYLPDWLEDTLSEGIRQWWKLKPGPPPPKPAERHKDDSRGLVLPGYKYLGPFNGLDKGEPVNEADAAALEHDKAYDRQLDSGDNPYLKYNHADAEFQERLKEDTSFGGNLGRAVFQAKKRVLEPLGLVEEPVKTAPGKKRPVEHSPVEPDSSSGTGKAGQQPARKRLNFGQTGDADSVPDPQPLGQPPAAPSGLGTNTMATGSGAPMADNNEGADGVGNSSGNWHCDSTWMGDRVITTSTRTWALPTYNNHLYKQISSQSGASNDNHYFGYSTPWGYFDFNRFHCHFSPRDWQRLINNNWGFRPKRLNFKLFNIQVKEVTQNDGTTTIANNLTSTVQVFTDSEYQLPYVLGSAHQGCLPPFPADVFMVPQYGYLTLNNGSQAVGRSSFYCLEYFPSQMLRTGNNFTFSYTFEDVPFHSSYAHSQSLDRLMNPLIDQYLYYLSRTNTPSGTTTQSRLQFSQAGASDIRDQSRNWLPGPCYRQQRVSKTSADNNNSEYSWTGATKYHLNGRDSLVNPGPAMASHKDDEEKFFPQSGVLIFGKQGSEKTNVDIEKVMITDEEEIRTTNPVATEQYGSVSTNLQRGNAAARGDLATLAARQAATADVNTQGVLPGMVWQDRDVYLQGPIWAKIPHTDGHFHPSPLMGGFGLKHPPPQILIKNTPVPANPSTTFSAAKFASFITQYSTGQVSVEIEWELQKENSKRWNPEIQYTSNYNKSVNVDFTVDTNGVYSEPRPIGTRYLTRNL

SEQ ID NO: 21 - protein, 747 aa, synthetic construct
MAADGYLPDWLEDTLSEGIRQWWKLKPGPPPPKPAERHKDDSRGLVLPGYKYLGPFNGLDKGEPVNEADAAALEHDKAYDRQLDSGDNPYLKYNHADAEFQERLKEDTSFGGNLGRAVFQAKKRVLEPLGLVEEPVKTAPGKKRPVEHSPVEPDSSSGTGKAGQQPARKRLNFGQTGDADSVPDPQPLGQPPAAPSGLGTNTMATGSGAPMADNNEGADGVGNSSGNWHCDSTWMGDRVITTSTRTWALPTYNNHLYKQISSQSGASNDNHYFGYSTPWGYFDFNRFHCHFSPRDWQRLINNNWGFRPKRLNFKLFNIQVKEVTQNDGTTTIANNLTSTVQVFTDSEYQLPYVLGSAHQGCLPPFPADVFMVPQYGYLTLNNGSQAVGRSSFYCLEYFPSQMLRTGNNFTFSYTFEDVPFHSSYAHSQSLDRLMNPLIDQYLYYLSRTNTPSGTTTQSRLQFSQAGASDIRDQSRNWLPGPCYRQQRVSKTSADNNNSEYSWTGATKYHLNGRDSLVNPGPAMASHKDDEEKFFPQSGVLIFGKQGSEKTNVDIEKVMITDEEEIRTTNPVATEQYGSVSTNLQRGNAAARGDLATPAARQAATADVNTQGVLPGMVWQDRDVYLQGPIWAKIPHTDGHFHPSPLMGGFGLKHPPPQILIKNTPVPANPSTTFSAAKFASFITQYSTGQVSVEIEWELQKENSKRWNPEIQYTSNYNKSVNVDFTVDTNGVYSEPRPIGTRYLTRNL

SEQ ID NO: 22 - protein, 747 aa, synthetic construct
MAADGYLPDWLEDTLSEGIRQWWKLKPGPPPPKPAERHKDDSRGLVLPGYKYLGPFNGLDKGEPVNEADAAALEHDKAYDRQLDSGDNPYLKYNHADAEFQERLKEDTSFGGNLGRAVFQAKKRVLEPLGLVEEPVKTAPGKKRPVEHSPVEPDSSSGTGKAGQQPARKRLNFGQTGDADSVPDPQPLGQPPAAPSGLGTNTMATGSGAPMADNNEGADGVGNSSGNWHCDSTWMGDRVITTSTRTWALPTYNNHLYKQISSQSGASNDNHYFGYSTPWGYFDFNRFHCHFSPRDWQRLINNNWGFRPKRLNFKLFNIQVKEVTQNDGTTTIANNLTSTVQVFTDSEYQLPYVLGSAHQGCLPPFPADVFMVPQYGYLTLNNGSQAVGRSSFYCLEYFPSQMLRTGNNFTFSYTFEDVPFHSSYAHSQSLDRLMNPLIDQYLYYLSRTNTPSGTTTQSRLQFSQAGASDIRDQSRNWLPGPCYRQQRVSKTSADNNNSEYSWTGATKYHLNGRDSLVNPGPAMASHKDDEEKFFPQSGVLIFGKQGSEKTNVDIEKVMITDEEEIRTTNPVATEQYGSVSTNLQRGNAAARGDLGRPAARQAATADVNTQGVLPGMVWQDRDVYLQGPIWAKIPHTDGHFHPSPLMGGFGLKHPPPQILIKNTPVPANPSTTFSAAKFASFITQYSTGQVSVEIEWELQKENSKRWNPEIQYTSNYNKSVNVDFTVDTNGVYSEPRPIGTRYLTRNL

SEQ ID NO: 23 - protein, 747 aa, synthetic construct
MAADGYLPDWLEDTLSEGIRQWWKLKPGPPPPKPAERHKDDSRGLVLPGYKYLGPFNGLDKGEPVNEADAAALEHDKAYDRQLDSGDNPYLKYNHADAEFQERLKEDTSFGGNLGRAVFQAKKRVLEPLGLVEEPVKTAPGKKRPVEHSPVEPDSSSGTGKAGQQPARKRLNFGQTGDADSVPDPQPLGQPPAAPSGLGTNTMATGSGAPMADNNEGADGVGNSSGNWHCDSTWMGDRVITTSTRTWALPTYNNHLYKQISSQSGASNDNHYFGYSTPWGYFDFNRFHCHFSPRDWQRLINNNWGFRPKRLNFKLFNIQVKEVTQNDGTTTIANNLTSTVQVFTDSEYQLPYVLGSAHQGCLPPFPADVFMVPQYGYLTLNNGSQAVGRSSFYCLEYFPSQMLRTGNNFTFSYTFEDVPFHSSYAHSQSLDRLMNPLIDQYLYYLSRTNTPSGTTTQSRLQFSQAGASDIRDQSRNWLPGPCYRQQRVSKTSADNNNSEYSWTGATKYHLNGRDSLVNPGPAMASHKDDEEKFFPQSGVLIFGKQGSEKTNVDIEKVMITDEEEIRTTNPVATEQYGSVSTNLQRGNAAARGDLGTLAARQAATADVNTQGVLPGMVWQDRDVYLQGPIWAKIPHTDGHFHPSPLMGGFGLKHPPPQILIKNTPVPANPSTTFSAAKFASFITQYSTGQVSVEIEWELQKENSKRWNPEIQYTSNYNKSVNVDFTVDTNGVYSEPRPIGTRYLTRNL

SEQ ID NO: 24 - protein, 747 aa, synthetic construct
MAADGYLPDWLEDTLSEGIRQWWKLKPGPPPPKPAERHKDDSRGLVLPGYKYLGPFNGLDKGEPVNEADAAALEHDKAYDRQLDSGDNPYLKYNHADAEFQERLKEDTSFGGNLGRAVFQAKKRVLEPLGLVEEPVKTAPGKKRPVEHSPVEPDSSSGTGKAGQQPARKRLNFGQTGDADSVPDPQPLGQPPAAPSGLGTNTMATGSGAPMADNNEGADGVGNSSGNWHCDSTWMGDRVITTSTRTWALPTYNNHLYKQISSQSGASNDNHYFGYSTPWGYFDFNRFHCHFSPRDWQRLINNNWGFRPKRLNFKLFNIQVKEVTQNDGTTTIANNLTSTVQVFTDSEYQLPYVLGSAHQGCLPPFPADVFMVPQYGYLTLNNGSQAVGRSSFYCLEYFPSQMLRTGNNFTFSYTFEDVPFHSSYAHSQSLDRLMNPLIDQYLYYLSRTNTPSGTTTQSRLQFSQAGASDIRDQSRNWLPGPCYRQQRVSKTSADNNNSEYSWTGATKYHLNGRDSLVNPGPAMASHKDDEEKFFPQSGVLIFGKQGSEKTNVDIEKVMITDEEEIRTTNPVATEQYGSVSTNLQRGNAAARGDLARIAARQAATADVNTQGVLPGMVWQDRDVYLQGPIWAKIPHTDGHFHPSPLMGGFGLKHPPPQILIKNTPVPANPSTTFSAAKFASFITQYSTGQVSVEIEWELQKENSKRWNPEIQYTSNYNKSVNVDFTVDTNGVYSEPRPIGTRYLTRNL

SEQ ID NO: 25 - protein, 747 aa, synthetic construct
MAADGYLPDWLEDTLSEGIRQWWKLKPGPPPPKPAERHKDDSRGLVLPGYKYLGPFNGLDKGEPVNEADAAALEHDKAYDRQLDSGDNPYLKYNHADAEFQERLKEDTSFGGNLGRAVFQAKKRVLEPLGLVEEPVKTAPGKKRPVEHSPVEPDSSSGTGKAGQQPARKRLNFGQTGDADSVPDPQPLGQPPAAPSGLGTNTMATGSGAPMADNNEGADGVGNSSGNWHCDSTWMGDRVITTSTRTWALPTYNNHLYKQISSQSGASNDNHYFGYSTPWGYFDFNRFHCHFSPRDWQRLINNNWGFRPKRLNFKLFNIQVKEVTQNDGTTTIANNLTSTVQVFTDSEYQLPYVLGSAHQGCLPPFPADVFMVPQYGYLTLNNGSQAVGRSSFYCLEYFPSQMLRTGNNFTFSYTFEDVPFHSSYAHSQSLDRLMNPLIDQYLYYLSRTNTPSGTTTQSRLQFSQAGASDIRDQSRNWLPGPCYRQQRVSKTSADNNNSEYSWTGATKYHLNGRDSLVNPGPAMASHKDDEEKFFPQSGVLIFGKQGSEKTNVDIEKVMITDEEEIRTTNPVATEQYGSVSTNLQRGNAAARGSLQNIAARQAATADVNTQGVLPGMVWQDRDVYLQGPIWAKIPHTDGHFHPSPLMGGFGLKHPPPQILIKNTPVPANPSTTFSAAKFASFITQYSTGQVSVEIEWELQKENSKRWNPEIQYTSNYNKSVNVDFTVDTNGVYSEPRPIGTRYLTRNL

SEQ ID NO: 26 - protein, 747 aa, synthetic construct
MAADGYLPDWLEDTLSEGIRQWWKLKPGPPPPKPAERHKDDSRGLVLPGYKYLGPFNGLDKGEPVNEADAAALEHDKAYDRQLDSGDNPYLKYNHADAEFQERLKEDTSFGGNLGRAVFQAKKRVLEPLGLVEEPVKTAPGKKRPVEHSPVEPDSSSGTGKAGQQPARKRLNFGQTGDADSVPDPQPLGQPPAAPSGLGTNTMATGSGAPMADNNEGADGVGNSSGNWHCDSTWMGDRVITTSTRTWALPTYNNHLYKQISSQSGASNDNHYFGYSTPWGYFDFNRFHCHFSPRDWQRLINNNWGFRPKRLNFKLFNIQVKEVTQNDGTTTIANNLTSTVQVFTDSEYQLPYVLGSAHQGCLPPFPADVFMVPQYGYLTLNNGSQAVGRSSFYCLEYFPSQMLRTGNNFTFSYTFEDVPFHSSYAHSQSLDRLMNPLIDQYLYYLSRTNTPSGTTTQSRLQFSQAGASDIRDQSRNWLPGPCYRQQRVSKTSADNNNSEYSWTGATKYHLNGRDSLVNPGPAMASHKDDEEKFFPQSGVLIFGKQGSEKTNVDIEKVMITDEEEIRTTNPVATEQYGSVSTNLQRGNAAARGSLQNLAARQAATADVNTQGVLPGMVWQDRDVYLQGPIWAKIPHTDGHFHPSPLMGGFGLKHPPPQILIKNTPVPANPSTTFSAAKFASFITQYSTGQVSVEIEWELQKENSKRWNPEIQYTSNYNKSVNVDFTVDTNGVYSEPRPIGTRYLTRNL

SEQ ID NO: 27 - protein, 744 aa, synthetic construct
MAADGYLPDWLEDTLSEGIRQWWKLKPGPPPPKPAERHKDDSRGLVLPGYKYLGPFNGLDKGEPVNEADAAALEHDKAYDRQLDSGDNPYLKYNHADAEFQERLKEDTSFGGNLGRAVFQAKKRVLEPLGLVEEPVKTAPGKKRPVEHSPVEPDSSSGTGKAGQQPARKRLNFGQTGDADSVPDPQPLGQPPAAPSGLGTNTMATGSGAPMADNNEGADGVGNSSGNWHCDSTWMGDRVITTSTRTWALPTYNNHLYKQISSQSGASNDNHYFGYSTPWGYFDFNRFHCHFSPRDWQRLINNNWGFRPKRLNFKLFNIQVKEVTQNDGTTTIANNLTSTVQVFTDSEYQLPYVLGSAHQGCLPPFPADVFMVPQYGYLTLNNGSQAVGRSSFYCLEYFPSQMLRTGNNFTFSYTFEDVPFHSSYAHSQSLDRLMNPLIDQYLYYLSRTNTPSGTTTQSRLQFSQAGASDIRDQSRNWLPGPCYRQQRVSKTSADNNNSEYSWTGATKYHLNGRDSLVNPGPAMASHKDDEEKFFPQSGVLIFGKQGSEKTNVDIEKVMITDEEEIRTTNPVATEQYGSVSTNLQRGNAAARGSLAARQAATADVNTQGVLPGMVWQDRDVYLQGPIWAKIPHTDGHFHPSPLMGGFGLKHPPPQILIKNTPVPANPSTTFSAAKFASFITQYSTGQVSVEIEWELQKENSKRWNPEIQYTSNYNKSVNVDFTVDTNGVYSEPRPIGTRYLTRNL

SEQ ID NO: 28 - protein, 735 aa, synthetic construct
MAADGYLPDWLEDTLSEGIRQWWKLKPGPPPPKPAERHKDDSRGLVLPGYKYLGPFNGLDKGEPVNEADAAALEHDKAYDRQLDSGDNPYLKYNHADAEFQERLKEDTSFGGNLGRAVFQAKKRVLEPLGLVEEPVKTAPGKKRPVEHSPVEPDSSSGTGKAGQQPARKRLNFGQTGDADSVPDPQPLGQPPAAPSGLGTNTMATGSGAPMADNNEGADGVGNSSGNWHCDSTWMGDRVITTSTRTWALPTYNNHLYKQISSQSGASNDNHYFGYSTPWGYFDFNRFHCHFSPRDWQRLINNNWGFRPKRLNFKLFNIQVKEVTQNDGTTTIANNLTSTVQVFTDSEYQLPYVLGSAHQGCLPPFPADVFMVPQYGYLTLNNGSQAVGRSSFYCLEYFPSQMLRTGNNFTFSYTFEDVPFHSSYAHSQSLDRLMNPLIDQYLYYLSRTNTPSGTTTQSRLQFSQAGASDIRDQSRNWLPGPCYRQQRVSKTSADNNNSEYSWTGATKYHLNGRDSLVNPGPAMASHKDDEEKFFPQSGVLIFGKQGSEKTNVDIEKVMITDEEEIRTTNPVATEQYGSVSTNLQRNGRQAATADVNTQGVLPGMVWQDRDVYLQGPIWAKIPHTDGHFHPSPLMGGFGLKHPPPQILIKNTPVPANPSTTFSAAKFASFITQYSTGQVSVEIEWELQKENSKRWNPEIQYTSNYNKSVNVDFTVDTNGVYSEPRPIGTRYLTRNL

SEQ ID NO: 29 - protein, 747 aa, synthetic construct
MAADGYLPDWLEDTLSEGIRQWWKLKPGPPPPKPAERHKDDSRGLVLPGYKYLGPFNGLDKGEPVNEADAAALEHDKAYDRQLDSGDNPYLKYNHADAEFQERLKEDTSFGGNLGRAVFQAKKRVLEPLGLVEEPVKTAPGKKRPVEHSPVEPDSSSGTGKAGQQPARKRLNFGQTGDADSVPDPQPLGQPPAAPSGLGTNTMATGSGAPMADNNEGADGVGNSSGNWHCDSTWMGDRVITTSTRTWALPTYNNHLYKQISSQSGASNDNHYFGYSTPWGYFDFNRFHCHFSPRDWQRLINNNWGFRPKRLNFKLFNIQVKEVTQNDGTTTIANNLTSTVQVFTDSEYQLPYVLGSAHQGCLPPFPADVFMVPQYGYLTLNNGSQAVGRSSFYCLEYFPSQMLRTGNNFTFSYTFEDVPFHSSYAHSQSLDRLMNPLIDQYLYYLSRTNTPSGTTTQSRLQFSQAGASDIRDQSRNWLPGPCYRQQRVSKTSADNNNSEYSWTGATKYHLNGRDSLVNPGPAMASHKDDEEKFFPQSGVLIFGKQGSEKTNVDIEKVMITDEEEIRTTNPVATEQYGSVSTNLQRGNAAAGNGRAHAAARQAATADVNTQGVLPGMVWQDRDVYLQGPIWAKIPHTDGHFHPSPLMGGFGLKHPPPQILIKNTPVPANPSTTFSAAKFASFITQYSTGQVSVEIEWELQKENSKRWNPEIQYTSNYNKSVNVDFTVDTNGVYSEPRPIGTRYLTRNL

SEQ ID NO: 30 - DNA, 60 bp, synthetic construct
  source 1..60: mol_type = other DNA
agcggctattgtagccagatcacctctggcagcagcgttgcctctctggaggttggtaga

SEQ ID NO: 31 - DNA, 60 bp, synthetic construct
  source 1..60: mol_type = other DNA
gctgctgccagaggtgatctggctacaatagccgctagacaagcagctaccgcagatgtc

SEQ ID NO: 32 - DNA, 63 bp, synthetic construct
  source 1..63: mol_type = other DNA
tgcagcgaggcgtcccaaatctcctctggctgcagcgttgcctctctggaggttggtagatac

SEQ ID NO: 33 - DNA, 63 bp, synthetic construct
  source 1..63: mol_type = other DNA
gctgcagccagaggagatttgggacgcctcgctgcaagacaagcagctaccgcagatgtcaac

SEQ ID NO: 34 - DNA, 65 bp, synthetic construct
  source 1..65: mol_type = other DNA
tgctgcaatattctgcaaatcacctcgggcagcggcgttgcctctctggaggttggtagatacag

SEQ ID NO: 35 - DNA, 65 bp, synthetic construct
  source 1..65: mol_type = other DNA
gccgctgcccgaggtgatttgcagaatattgcagcaagacaagcagctaccgcagatgtcaacac

SEQ ID NO: 36 - DNA, 65 bp, synthetic construct
  source 1..65: mol_type = other DNA
agctgccaaattctggaggtcacctcttgccgcagcgttgcctctctggaggttggtagatacag

SEQ ID NO: 37 - DNA, 65 bp, synthetic construct
  source 1..65: mol_type = other DNA
gctgcggcaagaggtgacctccagaatttggcagctagacaagcagctaccgcagatgtcaacac

SEQ ID NO: 38 - DNA, 65 bp, synthetic construct
  source 1..65: mol_type = other DNA
ggcggcaattgctgccagatcacctctggctgcagcgttgcctctctggaggttggtagatacag

SEQ ID NO: 39 - DNA, 65 bp, synthetic construct
  source 1..65: mol_type = other DNA
gctgcagccagaggtgatctggcagcaattgccgccagacaagcagctaccgcagatgtcaacac

SEQ ID NO: 40 - DNA, 65 bp, synthetic construct
  source 1..65: mol_type = other DNA
cgctgccagggttgccaagtcgcctcttgcagctgcgttgcctctctggaggttggtagatacag

SEQ ID NO: 41 - DNA, 67 bp, synthetic construct
  source 1..67: mol_type = other DNA
gcagctgcaagaggcgacttggcaaccctggcagcgagacaagcagctaccgcagatgtcaacacac

SEQ ID NO: 42 - DNA, 65 bp, synthetic construct
  source 1..65: mol_type = other DNA
ggcggctggcgttgccaaatcacccctagcagccgcgttgcctctctggaggttggtagatacag

SEQ ID NO: 43 - DNA, 65 bp, synthetic construct
  source 1..65: mol_type = other DNA
gcggctgctaggggtgatttggcaacgccagccgccagacaagcagctaccgcagatgtcaacac

SEQ ID NO: 44 - DNA, 65 bp, synthetic construct
  source 1..65: mol_type = other DNA
agctgcgggtctacccaaatcaccgcgggctgctgcgttgcctctctggaggttggtagatacag

SEQ ID NO: 45 - DNA, 65 bp, synthetic construct
  source 1..65: mol_type = other DNA
gcagcagcccgcggtgatttgggtagacccgcagctagacaagcagctaccgcagatgtcaacac

SEQ ID NO: 46 - DNA, 65 bp, synthetic construct
  source 1..65: mol_type = other DNA
cgcagcaagtgtaccaaggtctcctctggctgctgcgttgcctctctggaggttggtagatacag

SEQ ID NO: 47 - DNA, 67 bp, synthetic construct
  source 1..67: mol_type = other DNA
gcagcagccagaggagaccttggtacacttgctgcgagacaagcagctaccgcagatgtcaacacac

SEQ ID NO: 48 - DNA, 65 bp, synthetic construct
  source 1..65: mol_type = other DNA
tgctgcaatccttgcgaggtcacctcttgcagccgcgttgcctctctggaggttggtagatacag

SEQ ID NO: 49 - DNA, 65 bp, synthetic construct
  source 1..65: mol_type = other DNA
gcggctgcaagaggtgacctcgcaaggattgcagcaagacaagcagctaccgcagatgtcaacac

SEQ ID NO: 50 - DNA, 65 bp, synthetic construct
  source 1..65: mol_type = other DNA
agcggctatattttgcaggctgcctctcgcagcagcgttgcctctctggaggttggtagatacag

SEQ ID NO: 51 - DNA, 65 bp, synthetic construct
  source 1..65: mol_type = other DNA
gctgctgcgagaggcagcctgcaaaatatagccgctagacaagcagctaccgcagatgtcaacac

SEQ ID NO: 52 - DNA, 65 bp, synthetic construct
  source 1..65: mol_type = other DNA
ggcagccagattttggagagatcctcgtgctgctgcgttgcctctctggaggttggtagatacag

SEQ ID NO: 53 - DNA, 65 bp, synthetic construct
  source 1..65: mol_type = other DNA
gcagcagcacgaggatctctccaaaatctggctgccagacaagcagctaccgcagatgtcaacac

SEQ ID NO: 54 - DNA, 66 bp, synthetic construct
  source 1..66: mol_type = other DNA
tgccgcaagactgcccctagcagcggcgttgcctctctggaggttggtagatacagaaccatactg

SEQ ID NO: 55 - DNA, 64 bp, synthetic construct
  source 1..64: mol_type = other DNA
gccgctgctaggggcagtcttgcggcaagacaagcagctaccgcagatgtcaacacacaaggcg

SEQ ID NO: 56 - DNA, 45 bp, synthetic construct
  source 1..45: mol_type = other DNA
cggtagctgcttgtctgccgtttctctggaggttggtagatacag

SEQ ID NO: 57 - DNA, 42 bp, synthetic construct
  source 1..42: mol_type = other DNA
aacctccagagaaacggcagacaagcagctaccgcagatgtc

SEQ ID NO: 58 - DNA, 65 bp, synthetic construct
  source 1..65: mol_type = other DNA
ggctgctgcatgggcccgtccgtttcctgctgctgcgttgcctctctggaggttggtagatacag

SEQ ID NO: 59 - DNA, 65 bp, synthetic construct
  source 1..65: mol_type = other DNA
gcagcagcaggaaacggacgggcccatgcagcagccagacaagcagctaccgcagatgtcaacac

SEQ ID NO: 60 - protein, 735 aa, adeno-associated virus [sequence omitted]

SEQ ID NO: 61 - protein, 598 aa, adeno-associated virus
MAPGKKRPVEHSPVEPDSSSGTGKAGQQPARKRLNFGQTGDADSVPDPQPLGQPPAAPSGLGTNTMATGSGAPMADNNEGADGVGNSSGNWHCDSTWMGDRVITTSTRTWALPTYNNHLYKQISSQSGASNDNHYFGYSTPWGYFDFNRFHCHFSPRDWQRLINNNWGFRPKRLNFKLFNIQVKEVTQNDGTTTIANNLTSTVQVFTDSEYQLPYVLGSAHQGCLPPFPADVFMVPQYGYLTLNNGSQAVGRSSFYCLEYFPSQMLRTGNNFTFSYTFEDVPFHSSYAHSQSLDRLMNPLIDQYLYYLSRTNTPSGTTTQSRLQFSQAGASDIRDQSRNWLPGPCYRQQRVSKTSADNNNSEYSWTGATKYHLNGRDSLVNPGPAMASHKDDEEKFFPQSGVLIFGKQGSEKTNVDIEKVMITDEEEIRTTNPVATEQYGSVSTNLQRGNRQAATADVNTQGVLPGMVWQDRDVYLQGPIWAKIPHTDGHFHPSPLMGGFGLKHPPPQILIKNTPVPANPSTTFSAAKFASFITQYSTGQVSVEIEWELQKENSKRWNPEIQYTSNYNKSVNVDFTVDTNGVYSEPRPIGTRYLTRNL

SEQ ID NO: 62 - protein, 533 aa, adeno-associated virus
MATGSGAPMADNNEGADGVGNSSGNWHCDSTWMGDRVITTSTRTWALPTYNNHLYKQISSQSGASNDNHYFGYSTPWGYFDFNRFHCHFSPRDWQRLINNNWGFRPKRLNFKLFNIQVKEVTQNDGTTTIANNLTSTVQVFTDSEYQLPYVLGSAHQGCLPPFPADVFMVPQYGYLTLNNGSQAVGRSSFYCLEYFPSQMLRTGNNFTFSYTFEDVPFHSSYAHSQSLDRLMNPLIDQYLYYLSRTNTPSGTTTQSRLQFSQAGASDIRDQSRNWLPGPCYRQQRVSKTSADNNNSEYSWTGATKYHLNGRDSLVNPGPAMASHKDDEEKFFPQSGVLIFGKQGSEKTNVDIEKVMITDEEEIRTTNPVATEQYGSVSTNLQRGNRQAATADVNTQGVLPGMVWQDRDVYLQGPIWAKIPHTDGHFHPSPLMGGFGLKHPPPQILIKNTPVPANPSTTFSAAKFASFITQYSTGQVSVEIEWELQKENSKRWNPEIQYTSNYNKSVNVDFTVDTNGVYSEPRPIGTRYLTRNL

SEQ ID NO: 63 - DNA, 7493 bp, synthetic construct
  source 1..7493: mol_type = other DNA
gcgcgccgatatcttcaaacctcccgcttcaaaatggagaccctgcgtgctcactcgggcccccccccccagcgtgaccacatggtgtcgcaaaatgtcgcaaaacactcacgtgacctctaatacaggacctccctaaccctatgacgtaattcacgtcacgactccacccctccgttaacgccccgcgccggccgctctagaactagtggatcccccggaagatcagaagttcctattccgaagttcctattctctagaaagtataggaacttctgatctgcgcagccgccatgccggggttttacgagattgtgattaaggtccccagcgaccttgacgagcatctgcccggcatttctgacagctttgtgaactgggtggccgagaaggaatgggagttgccgccagattctgacatggatctgaatctgattgagcaggcacccctgaccgtggccgagaagctgcagcgcgactttctgacggaatggcgccgtgtgagtaaggccccggaggcccttttctttgtgcaatttgagaagggagagagctacttccacatgcacgtgctcgtggaaaccaccggggtgaaatccatggttttgggacgtttcctgagtcagattcgcgaaaaactgattcagagaatttaccgcgggatcgagccgactttgccaaactggttcgcggtcacaaagaccagaaatggcgccggaggcgggaacaaggtggtggatgagtgctacatccccaattacttgctccccaaaacccagcctgagctccagtgggcgtggactaatatggaacagtatttaagcgcctgtttgaatctcacggagcgtaaacggttggtggcgcagcatctgacgcacgtgtcgcagacgcaggagcagaacaaagagaatcagaatcccaattctgatgcgccggtgatcagatcaaaaacttcagccaggtacatggagctggtcgggtggctcgtggacaaggggattacctcggagaagcagtggatccaggaggaccaggcctcatacatctccttcaatgcggcctccaactcgcggtcccaaatcaaggctgccttggacaatgcgggaaagattatgagcctgactaaaaccgcccccgactacctggtgggccagcagcccgtggaggacatttccagcaatcggatttataaaattttggaactaaacgggtacgatccccaatatgcggcttccgtctttctgggatgggccacgaaaaagttcggcaagaggaacaccatctggctgtttgggcctgcaactaccgggaagaccaacatcgcggaggccatagcccacactgtgcccttctacgggtgcgtaaactggaccaatgagaactttcccttcaacgactgtgtcgacaagatggtgatctggtgggaggaggggaagatgaccgccaaggtcgtggagtcggccaaagccattctcggaggaagcaaggtgcgcgtggaccagaaatgcaagtcctcggcccagatagacccgactcccgtgatcgtcacctccaacaccaacatgtgcgccgtgattgacgggaactcaacgaccttcgaacaccagcagccgttgcaagaccggatgttcaaatttgaactcacccgccgtctggatcatgactttgggaaggtcaccaagcaggaagtcaaagactttttccggtgggcaaaggatcacgtggttgaggtggagcatgaattctacgtcaaaaagggtggagccaagaaaagacccgcccccagtgacgcagatataagtgagcccaaacgggtgcgcgagtcagttgcgcagccatcgacgtcagacgcggaagcttcgatcaactacgcagacaggtaccaaaacaaatgttctcgtcacgtgggcatgaatctgatgctgtttccctgcagacaatgcgagagaatgaatcagaattcaaatatctgcttcactcacggacagaaagactgtttagagtgctttcccgtgtcagaatctcaacccgtttctgtcgtcaaaaaggcgtatcagaaactgtgctacattcatcatatcatgggaaaggtgccagacgcttgcactgcctgcgatctggtcaatgtggatttggatgactgcatctttgaacaataaatgatttaaatcaggtatggctgccgatggttatcttccagattggctcgaggacactctctctgaaggaataagacagtggtggaagctcaaacctggcccaccaccaccaaagcccgcagagcggcataaggacgacagcaggggtcttgtgcttcctgggtacaagtacctcggacccttcaacggactcgacaagggagagccggtcaacgaggcagacgccgcggccctcgagcacgacaaagcctacgaccggcagctcgacagcggagacaacccgtacctcaagtacaaccacgccgacgcggagtttcaggagcgccttaaagaagatacgtcttttgggggcaacctcggacgagcagtcttccaggcgaaaaagagggttcttgaacctctgggcctggttgaggaacctgttaagacggctccgggaaaaaagaggccggtagagcactctcctgtggagccagactcctcctcgggaaccggaaaggcgggccagcagcctgcaagaaaaagattgaattttggtcagactggagacgcagactcagtacctgacccccagcctctcggacagccaccagcagccccctctggtctgggaactaatacgatggctacaggcagtggcgcaccaatggcagacaataacgagggcgccgacggagtgggtaattcctcgggaaattggcattgcgattccacatggatgggcgacagagtcatcaccaccagcacccgaacctgggccctgcccacctacaacaaccacctctacaaacaaatttccagccaatcaggagcctcgaacgacaatcactactttggctacagcaccccttgggggtattttgacttcaacagattccactgccacttttcaccacgtgactggcaaagactcatcaacaacaactggggattccgacccaagagactcaacttcaagctctttaacattcaagtcaaagaggtcacgcagaatgacggtacgacgacgattgccaataaccttaccagcacggttcaggtgtttactgactcggagtaccagctcccgtacgtcctcggctcggcgcatcaaggatgcctcccgccgttcccagcagacgtcttcatggtgccacagtatggatacctcaccctgaacaacgggagtcaggcagtaggacgctcttcattttactgcctggagtactttccttctcagatgctgcgtaccggaaacaactttaccttcagctacacttttgaggacgttcctttccacagcagctacgctcacagccagagtctggaccgtctcatgaatcctctcatcgaccagtacctgtattacttgagcagaacaaacactccaagtggaaccaccacgcagtcaaggcttcagttttctcaggccggagcgagtgacattcgggaccagtctaggaactggcttcctggaccctgttaccgccagcagcgagtatcaaagacatctgcggataacaacaacagtgaatactcgtggactggagctaccaagtaccacctcaatggcagagactctctggtgaatccgggcccggccatggcaagccacaaggacgatgaagaaaagttttttcctcagagcggggttctcatctttgggaagcaaggctcagagaaaacaaatgtggacattgaaaaggtcatgattacagacgaagaggaaatcaggacaaccaatcccgtggctacggagcagtatggttctgtatctaccaacctccagcgcggccgcaacagacaagcagctaccgcagatgtcaacacacaaggcgttcttccaggcatggtctggcaggacagagatgtgtaccttcaggggcccatctgggcaaagattccacacacggacggacattttcacccctctcccctcatgggtggattcggacttaaacaccctcctccacagattctcatcaagaacaccccggtacctgcgaatccttcgaccaccttcagtgcggcaaagtttgcttccttcatcacacagtactccacgggacaggtcagcgtggagatcgagtgggagctgcagaaggaaaacagcaaacgctggaatcccgaaattcagtacacttccaactacaacaagtctgttaatgtggactttactgtggacactaatggcgtgtattcagagcctcgccccattggcaccagatacctgactcgtaatctgtaattgcttgttaatcaataaaccgtttaattcgtttcagttgaactttggtctctgcgtatttctttcttatctagtttccatggctacgtagataagtagcatggcgggttaatcattaactacagcccgggcgtttaaacagcgggcggaggggtggagtcgtgacgtgaattacgtcatagggttagggaggtcctgtattagaggtcacgtgagtgttttgcgacattttgcgacaccatgtggtctcgctgggggggggggcccgagtgagcacgcagggtctccattttgaagcgggaggtttgaacgagcgctggcgcgctcactggccgtcgttttacaacgtcgtgactgggaaaaccctggcgttacccaacttaatcgccttgcagcacatccccctttcgccagctggcgtaatagcgaagaggcccgcaccgatcgcccttcccaacagttgcgcagcctgaatggcgaatggaaattgtaagcgttaatattttgttaaaattcgcgttaaatttttgttaaatcagctcatttttttaaccaataggccgaaatcggcaaaatcccttataaatcaaaagaatagaccgagatagggttgagtgttgttccagtttggaacaagagtccactattaagaacgtggactccaacgtcaaagggcgaaaaaccgtctatcagggcgatggcccactacgtgaaccatcaccctaatcaagttttttggggtcgaggtgccgtaaagcactaaatcggaaccctaaagggagcccccgatttagagcttgacggggaaagccggcgaacgtggcgagaaaggaagggaagaaagcgaaaggagcgggcgctagggcgctggcaagtgtagcggtcacgctgcgcgtaaccaccacacccgccgcgcttaatgcgccgctacagggcgcgtcaggtggcacttttcggggaaatgtgcgcggaacccctatttgtttatttttctaaatacattcaaatatgtatccgctcatgagacaataaccctgataaatgcttcaataatattgaaaaaggaagagtatgagtattcaacatttccgtgtcgcccttattcccttttttgcggcattttgccttcctgtttttgctcacccagaaacgctggtgaaagtaaaagatgctgaagatcagttgggtgcacgagtgggttacatcgaactggatctcaacagcggtaagatccttgagagttttcgccccgaagaacgttttccaatgatgagcacttttaaagttctgctatgtggcgcggtattatcccgtattgacgccgggcaagagcaactcggtcgccgcatacactattctcagaatgacttggttgagtactcaccagtcacagaaaagcatcttacggatggcatgacagtaagagaattatgcagtgctgccataaccatgagtgataacactgcggccaacttacttctgacaacgatcggaggaccgaaggagctaaccgcttttttgcacaacatgggggatcatgtaactcgccttgatcgttgggaaccggagctgaatgaagccataccaaacgacgagcgtgacaccacgatgcctgtagcaatggcaacaacgttgcgcaaactattaactggcgaactacttactctagcttcccggcaacaattaatagactggatggaggcggataaagttgcaggaccacttctgcgctcggcccttccggctggctggtttattgctgataaatctggagccggtgagcgtgggtctcgcggtatcattgcagcactggggccagatggtaagccctcccgtatcgtagttatctacacgacggggagtcaggcaactatggatgaacgaaatagacagatcgctgagataggtgcctcactgattaagcattggtaactgtcagaccaagtttactcatatatactttagattgatttaaaacttcatttttaatttaaaaggatctaggtgaagatcctttttgataatctcatgaccaaaatcccttaacgtgagttttcgttccactgagcgtcagaccccgtagaaaagatcaaaggatcttcttgagatcctttttttctgcgcgtaatctgctgcttgcaaacaaaaaaaccaccgctaccagcggtggtttgtttgccggatcaagagctaccaactctttttccgaaggtaactggcttcagcagagcgcagataccaaatactgttcttctagtgtagccgtagttaggccaccacttcaagaactctgtagcaccgcctacatacctcgctctgctaatcctgttaccagtggctgctgccagtggcgataagtcgtgtcttaccgggttggactcaagacgatagttaccggataaggcgcagcggtcgggctgaacggggggttcgtgcacacagcccagcttggagcgaacgacctacaccgaactgagatacctacagcgtgagctatgagaaagcgccacgcttcccgaagggagaaaggcggacaggtatccggtaagcggcagggtcggaacaggagagcgcacgagggagcttccagggggaaacgcctggtatctttatagtcctgtcgggtttcgccacctctgacttgagcgtcgatttttgtgatgctcgtcaggggggcggagcctatggaaaaacgccagcaacgcggcctttttacggttcctggccttttgctggccttttgctcacatgttctttcctgcgttatcccctgattctgtggataaccgtattaccgcctttgagtgagctgataccgctcgccgcagccgaacgaccgagcgcagcgagtcagtgagcgaggaagcggaagagcgcccaatacgcaaaccgcctctccccgcgcgttggccgattcattaatgcagctggcacgacaggtttcccgactggaaagcgggcagtgagcgcaacgcaattaatgtgagttagctcactcattaggcaccccaggctttacactttatgcttccggctcgtatgttgtgtggaattgtgagcggataacaatttcacacaggaaacagctatgaccatgattacgccaa

SEQ ID NO: 64 - DNA, 7354 bp, synthetic construct
  source 1..7354: mol_type = other DNA
ttggtctctgcgaagggcgaattcgtttaaacctgcaggactagaggtcctgtattagaggtcacgtgagtgttttgcgacattttgcgacaccatgtggtcacgctgggtatttaagcccgagtgagcacgcagggtctccattttgaagcgggaggtttgaacgcgcagccgccaagccgaattctgcagatatccatcacactggcggccgctcgactagagcggccgccaccgcggtggagctccagcttttgttccctttagtgagggttaattgcgcgcttggcgtaatcatggtcatagctgtttcctgtgtgaaattgttatccgctcacaattccacacaacatacgagccggaagcataaagtgtaaagcctggggtgcctaatgagtgagctaactcacattaattgcgttgcgctcactgcccgctttccagtcgggaaacctgtcgtgccagctgcattaatgaatcggccaacgcgcggggagaggcggtttgcgtattgggcgctcttccgcttcctcgctcactgactcgctgcgctcggtcgttcggctgcggcgagcggtatcagctcactcaaaggcggtaatacggttatccacagaatcaggggataacgcaggaaagaacatgtgagcaaaaggccagcaaaaggccaggaaccgtaaaaaggccgcgttgctggcgtttttccataggctccgcccccctgacgagcatcacaaaaatcgacgctcaagtcagaggtggcgaaacccgacaggactataaagataccaggcgtttccccctggaagctccctcgtgcgctctcctgttccgaccctgccgcttaccggatacctgtccgcctttctcccttcgggaagcgtggcgctttctcatagctcacgctgtaggtatctcagttcggtgtaggtcgttcgctccaagctgggctgtgtgcacgaaccccccgttcagcccgaccgctgcgccttatccggtaactatcgtcttgagtccaacccggtaagacacgacttatcgccactggcagcagccactggtaacaggattagcagagcgaggtatgtaggcggtgctacagagttcttgaagtggtggcctaactacggctacactagaagaacagtatttggtatctgcgctctgctgaagccagttaccttcggaaaaagagttggtagctcttgatccggcaaacaaaccaccgctggtagcggtggtttttttgtttgcaagcagcagattacgcgcagaaaaaaaggatctcaagaagatcctttgatcttttctacggggtctgacgctcagtggaacgaaaactcacgttaagggattttggtcatgagattatcaaaaaggatcttcacctagatccttttaaattaaaaatgaagttttaaatcaatctaaagtatatatgagtaaacttggtctgacagttaccaatgcttaatcagtgaggcacctatctcagcgatctgtctatttcgttcatccatagttgcctgactccccgtcgtgtagataactacgatacgggagggcttaccatctggccccagtgctgcaatgataccgcgagacccacgctcaccggctccagatttatcagcaataaaccagccagccggaagggccgagcgcagaagtggtcctgcaactttatccgcctccatccagtctattaattgttgccgggaagctagagtaagtagttcgccagttaatagtttgcgcaacgttgttgccattgctacaggcatcgtggtgtcacgctcgtcgtttggtatggcttcattcagctccggttcccaacgatcaaggcgagttacatgatcccccatgttgtgcaaaaaagcggttagctccttcggtcctccgatcgttgtcagaagtaagttggccgcagtgttatcactcatggttatggcagcactgcataattctcttactgtcatgccatccgtaagatgcttttctgtgactggtgagtactcaaccaagtcattctgagaatagtgtatgcggcgaccgagttgctcttgcccggcgtcaatacgggataataccgcgccacatagcagaactttaaaagtgctcatcattggaaaacgttcttcggggcgaaaactctcaaggatcttaccgctgttgagatccagttcgatgtaacccactcgtgcacccaactgatcttcagcatcttttactttcaccagcgtttctgggtgagcaaaaacaggaaggcaaaatgccgcaaaaaagggaataagggcgacacggaaatgttgaatactcatactcttcctttttcaatattattgaagcatttatcagggttattgtctcatgagcggatacatatttgaatgtatttagaaaaataaacaaataggggttccgcgcacatttccccgaaaagtgccacctaaattgtaagcgttaatattttgttaaaattcgcgttaaatttttgttaaatcagctcattttttaaccaataggccgaaatcggcaaaatcccttataaatcaaaagaatagaccgagatagggttgagtgttgttccagtttggaacaagagtccactattaaagaacgtggactccaacgtcaaagggcgaaaaaccgtctatcagggcgatggcccactacgtgaaccatcaccctaatcaagttttttggggtcgaggtgccgtaaagcactaaatcggaaccctaaagggagcccccgatttagagcttgacggggaaagccggcgaacgtggcgagaaaggaagggaagaaagcgaaaggagcgggcgctagggcgctggcaagtgtagcggtcacgctgcgcgtaaccaccacacccgccgcgcttaatgcgccgctacagggcgcgtcccattcgccattcaggctgcgcaactgttgggaagggcgatcggtgcgggcctcttcgctattacgccagctggcgaaagggggatgtgctgcaaggcgattaagttgggtaacgccagggttttcccagtcacgacgttgtaaaacgacggccagtgagcgcgcgtaatacgactcactatagggcgaattgggtaccgggccccccctcgatcgaggtcgacggtatcgggggagctcgcagggtctccattttgaagcgggaggtttgaacgcgcagccgccatgccggggttttacgagattgtgattaaggtccccagcgaccttgacgagcatctgcccggcatttctgacagctttgtgaactgggtggccgagaaggaatgggagttgccgccagattctgacatggatctgaatctgattgagcaggcacccctgaccgtggccgagaagctgcagcgcgactttctgacggaatggcgccgtgtgagtaaggccccggaggcccttttctttgtgcaatttgagaagggagagagctacttccacatgcacgtgctcgtggaaaccaccggggtgaaatccatggttttgggacgtttcctgagtcagattcgcgaaaaactgattcagagaatttaccgcgggatcgagccgactttgccaaactggttcgcggtcacaaagaccagaaatggcgccggaggcgggaacaaggtggtggatgagtgctacatccccaattacttgctccccaaaacccagcctgagctccagtgggcgtggactaatatggaacagtatttaagcgcctgtttgaatctcacggagcgtaaacggttggtggcgcagcatctgacgcacgtgtcgcagacgcaggagcagaacaaagagaatcagaatcccaattctgatgcgccggtgatcagatcaaaaacttcagccaggtacatggagctggtcgggtggctcgtggacaaggggattacctcggagaagcagtggatccaggaggaccaggcctcatacatctccttcaatgcggcctccaactcgcggtcccaaatcaaggctgccttggacaatgcgggaaagattatgagcctgactaaaaccgcccccgactacctggtgggccagcagcccgtggaggacatttccagcaatcggatttataaaattttggaactaaacgggtacgatccccaatatgcggcttccgtctttctgggatgggccacgaaaaagttcggcaagaggaacaccatctggctgtttgggcctgcaactaccgggaagaccaacatcgcggaggccatagcccacactgtgcccttctacgggtgcgtaaactggaccaatgagaactttcccttcaacgactgtgtcgacaagatggtgatctggtgggaggaggggaagatgaccgccaaggtcgtggagtcggccaaagccattctcggaggaagcaaggtgcgcgtggaccagaaatgcaagtcctcggcccagatagacccgactcccgtgatcgtcacctccaacaccaacatgtgcgccgtgattgacgggaactcaacgaccttcgaacaccagcagccgttgcaagaccggatgttcaaatttgaactcacccgccgtctggatcatgactttgggaaggtcaccaagcaggaagtcaaagactttttccggtgggcaaaggatcacgtggttgaggtggagcatgaattctacgtcaaaaagggtggagccaagaaaagacccgcccccagtgacgcagatataagtgagcccaaacgggtgcgcgagtcagttgcgcagccatcgacgtcagacgcggaagcttcgatcaactacgcagacaggtaccaaaacaaatgttctcgtcacgtgggcatgaatctgatgctgtttccctgcagacaatgcgagagaatgaatcagaattcaaatatctgcttcactcacggacagaaagactgtttagagtgctttcccgtgtcagaatctcaacccgtttctgtcgtcaaaaaggcgtatcagaaactgtgctacattcatcatatcatgggaaaggtgccagacgcttgcactgcctgcgatctggtcaatgtggatttggatgactgcatctttgaacaataaatgatttaaatcaggtatggctgccgatggttatcttccagattggctcgaggacactctctctgaaggaataagacagtggtggaagctcaaacctggcccaccaccaccaaaggccgcagagcggcataaggacgacagcaggggtcttgtgcttcctgggtacaagtacctcggacccttcaacggactcgacaagggagagccggtcaacgaggcagacgccgcggccctcgagcacgacaaagcctacgaccggcagctcgacagcggagacaacccgtacctcaagtacaaccacgccgacgcggagtttcaggagcgccttaaagaagatacgtcttttgggggcaacctcggacgagcagtcttccaggcgaaaaagagggttcttgaacctctgggcctggttgaggaacctgttaagacggctccgggaaaaaagaggccggtagagcactctcctgtggagccagactcctcctcgggaaccggaaaggcgggccagcagcctgcaagaaaaagattgaattttggtcagactggagacgcagactcagtacctgacccccagcctctcggacagccaccagcagccccctctggtctgggaactaatacgatggctacaggcagtggcgcaccaatggcagacaataacgagggcgccgacggagtgggtaattcctcgggaaattggcattgcgattccacatggatgggcgacagagtcatcaccaccagcacccgaacctgggccctgcccacctacaacaaccacctctacaaacaaatttccagccaatcaggagcctcgaacgacaatcactactttggctacagcaccccttgggggtattttgacttcaacagattccactgccacttttcaccacgtgactggcaaagactcatcaacaacaactggggattccgacccaagagactcaacttcaagctctttaacattcaagtcaaagaggtcacgcagaatgacggtacgacgacgattgccaataaccttaccagcacggttcaggtgtttactgactcggagtaccagctcccgtacgtcctcggctcggcgcatcaaggatgcctcccgccgttcccagcagacgtcttcatggtgccacagtatggatacctcaccctgaacaacgggagtcaggcagtaggacgctcttcattttactgcctggagtactttccttctcagatgctgcgtaccggaaacaactttaccttcagctacacttttgaggacgttcctttccacagcagctacgctcacagccagagtctggaccgtctcatgaatcctctcatcgaccagtacctgtattacttgagcagaacaaacactccaagtggaaccaccacgcagtcaaggcttcagttttctcaggccggagcgagtgacattcgggaccagtctaggaactggcttcctggaccctgttaccgccagcagcgagtatcaaagacatctgcggataacaacaacagtgaatactcgtggactggagctaccaagtaccacctcaatggcagagactctctggtgaatccgggcccggccatggcaagccacaaggacgatgaagaaaagttttttcctcagagcggggttctcatctttgggaagcaaggctcagagaaaacaaatgtggacattgaaaaggtcatgattacagacgaagaggaaatcaggacaaccaatcccgtggctacggagcagtatggttctgtatctaccaacctccagagaggcaacgccgctgctaggggcagtcttgcggcaagacaagcagctaccgcagatgtcaacacacaaggcgttcttccaggcatggtctggcaggacagagatgtgtaccttcaggggcccatctgggcaaagattccacacacggacggacattttcacccctctcccctcatgggtggattcggacttaaacaccctcctccacagattctcatcaagaacaccccggtacctgcgaatccttcgaccaccttcagtgcggcaaagtttgcttccttcatcacacagtactccacgggacaggtcagcgtggagatcgagtgggagctgcagaaggaaaacagcaaacgctggaatcccgaaattcagtacacttccaactacaacaagtctgttaatgtggactttactgtggacactaatggcgtgtattcagagcctcgccccattggcaccagatacctgactcgtaatctgtaattgcctgttaatcaataaaccggttgattcgtttcagttgaact

SEQ ID NO: 65 - protein, 744 aa, synthetic construct
MAADGYLPDWLEDTLSEGIRQWWKLKPGPPPPKAAERHKDDSRGLVLPGYKYLGPFNGLDKGEPVNEADAAALEHDKAYDRQLDSGDNPYLKYNHADAEFQERLKEDTSFGGNLGRAVFQAKKRVLEPLGLVEEPVKTAPGKKRPVEHSPVEPDSSSGTGKAGQQPARKRLNFGQTGDADSVPDPQPLGQPPAAPSGLGTNTMATGSGAPMADNNEGADGVGNSSGNWHCDSTWMGDRVITTSTRTWALPTYNNHLYKQISSQSGASNDNHYFGYSTPWGYFDFNRFHCHFSPRDWQRLINNNWGFRPKRLNFKLFNIQVKEVTQNDGTTTIANNLTSTVQVFTDSEYQLPYVLGSAHQGCLPPFPADVFMVPQYGYLTLNNGSQAVGRSSFYCLEYFPSQMLRTGNNFTFSYTFEDVPFHSSYAHSQSLDRLMNPLIDQYLYYLSRTNTPSGTTTQSRLQFSQAGASDIRDQSRNWLPGPCYRQQRVSKTSADNNNSEYSWTGATKYHLNGRDSLVNPGPAMASHKDDEEKFFPQSGVLIFGKQGSEKTNVDIEKVMITDEEEIRTTNPVATEQYGSVSTNLQRGNAAARGSLAARQAATADVNTQGVLPGMVWQDRDVYLQGPIWAKIPHTDGHFHPSPLMGGFGLKHPPPQILIKNTPVPANPSTTFSAAKFASFITQYSTGQVSVEIEWELQKENSKRWNPEIQYTSNYNKSVNVDFTVDTNGVYSEPRPIGTRYLTRNL

SEQ ID NO: 66 - protein, 14 aa, synthetic construct
QAGTFALRGDNPQG